European Patent Application EP 4 206 220 A1, published July 5, 2023. Title: Novel proinsulin glargine and method for preparing insulin glargine therefrom. Applicant: TANG, Chuangen WANG, Jing PAN, Shangshu FAN, Xiaoyang LIU, Xiaorui CHEN, Song ZHANG, Haoning. The sequence listing filed with the application follows.

SEQUENCE LISTING (22 sequences)

SEQ ID NO: 1 - protein, 64 aa, Artificial sequence
  Protein translated from synthetic DNA
MATKAVSVLKGDGPVQGIINFEQKESNGPVKVWGSIKGLTEGLHGFHVHEFGDNTAGSTSAGPR

SEQ ID NO: 2 - protein, 63 aa, Artificial sequence
  Protein translated from synthetic DNA
MATPAVSVLKGDGPVQGIINFEQPESNGPVKVWGSIPGLTEGLHGFHVHEFGDNTAGSTSAGP

SEQ ID NO: 3 - protein, 63 aa, Artificial sequence
  Protein translated from synthetic DNA
MATHAVSVLKGDGPVQGIINFEQHESNGPVKVWGSIHGLTEGLHGFHVHEFGDNTAGSTSAGP

SEQ ID NO: 4 - protein, 20 aa, Homo sapiens
GIVEQCCTSICSLYQLENYC

SEQ ID NO: 5 - protein, 30 aa, Homo sapiens
FVNQHLCGSHLVEALYLVCGERGFFYTPKT

SEQ ID NO: 6 - protein, 53 aa, Artificial sequence
  Protein translated from synthetic DNA
FVNQHLCGSHLVEALYLVCGERGFFYTPKTRRGIVEQCCTSICSLYQLENYCG

SEQ ID NO: 7 - protein, 117 aa, Artificial sequence
  Protein translated from synthetic DNA
MATPAVSVLKGDGPVQGIINFEQPESNGPVKVWGSIPGLTEGLHGFHVHEFGDNTAGSTSAGPKFVNQHLCGSHLVEALYLVCGERGFFYTPKTRRGIVEQCCTSICSLYQLENYCG

SEQ ID NO: 8 - protein, 117 aa, Artificial sequence
  Protein translated from synthetic DNA
MATPAVSVLKGDGPVQGIINFEQPESNGPVKVWGSIPGLTEGLHGFHVHEFGDNTAGSTSAGPRFVNQHLCGSHLVEALYLVCGERGFFYTPKTRRGIVEQCCTSICSLYQLENYCG

SEQ ID NO: 9 - protein, 117 aa, Artificial sequence
  Protein translated from synthetic DNA
MATHAVSVLKGDGPVQGIINFEQHESNGPVKVWGSIHGLTEGLHGFHVHEFGDNTAGSTSAGPKFVNQHLCGSHLVEALYLVCGERGFFYTPKTRRGIVEQCCTSICSLYQLENYCG

SEQ ID NO: 10 - protein, 117 aa, Artificial sequence
  Protein translated from synthetic DNA
MATHAVSVLKGDGPVQGIINFEQHESNGPVKVWGSIHGLTEGLHGFHVHEFGDNTAGSTSAGPRFVNQHLCGSHLVEALYLVCGERGFFYTPKTRRGIVEQCCTSICSLYQLENYCG

SEQ ID NO: 11 - DNA, 354 bp, Artificial sequence
  Synthetic DNA
atggcgacgccggccgtgagcgtgctgaagggcgacggcccagtgcagggcatcatcaatttcgagcagccggaaagtaatggaccagtgaaggtgtggggaagcattccgggactgactgaaggcctgcatggattccatgttcatgagtttggagataatacagctggctctaccagtgcaggtccgaaatttgtgaaccagcatctgtgcggcagccatctggtggaagcgctgtatctggtgtgcggcgaacgcggcttcttttataccccgaaaacccgccgcggcattgtggaacagtgctgcaccagcatttgcagcctgtatcagctggaaaactattgcggctaa

SEQ ID NO: 12 - DNA, 354 bp, Artificial sequence
  Synthetic DNA
atggcgacgccggccgtgagcgtgctgaagggcgacggcccagtgcagggcatcatcaatttcgagcagccggaaagtaatggaccagtgaaggtgtggggaagcattccgggactgactgaaggcctgcatggattccatgttcatgagtttggagataatacagctggctctaccagtgcaggtccgcggtttgtgaaccagcatctgtgcggcagccatctggtggaagcgctgtatctggtgtgcggcgaacgcggcttcttttataccccgaaaacccgccgcggcattgtggaacagtgctgcaccagcatttgcagcctgtatcagctggaaaactattgcggctaa

SEQ ID NO: 13 - DNA, 354 bp, Artificial sequence
  Synthetic DNA
atggcgacgcatgccgtgagcgtgctgaagggcgacggcccagtgcagggcatcatcaatttcgagcagcatgaaagtaatggaccagtgaaggtgtggggaagcattcatggactgactgaaggcctgcatggattccatgttcatgagtttggagataatacagctggctctaccagtgcaggtccgaaatttgtgaaccagcatctgtgcggcagccatctggtggaagcgctgtatctggtgtgcggcgaacgcggcttcttttataccccgaaaacccgccgcggcattgtggaacagtgctgcaccagcatttgcagcctgtatcagctggaaaactattgcggctaa

SEQ ID NO: 14 - DNA, 354 bp, Artificial sequence
  Synthetic DNA
atggcgacgcatgccgtgagcgtgctgaagggcgacggcccagtgcagggcatcatcaatttcgagcagcatgaaagtaatggaccagtgaaggtgtggggaagcattcatggactgactgaaggcctgcatggattccatgttcatgagtttggagataatacagctggctctaccagtgcaggtccgcggtttgtgaaccagcatctgtgcggcagccatctggtggaagcgctgtatctggtgtgcggcgaacgcggcttcttttataccccgaaaacccgccgcggcattgtggaacagtgctgcaccagcatttgcagcctgtatcagctggaaaactattgcggctaa

SEQ ID NO: 15 - protein, 117 aa, Artificial sequence
  Protein translated from synthetic DNA
MATKAVSVLKGDGPVQGIINFEQKESNGPVKVWGSIKGLTEGLHGFHVHEFGDNTAGSTSAGPKFVNQHLCGSHLVEALYLVCGERGFFYTPKTRRGIVEQCCTSICSLYQLENYCG

SEQ ID NO: 16 - protein, 117 aa, Artificial sequence
  Protein translated from synthetic DNA
MATKAVSVLKGDGPVQGIINFEQKESNGPVKVWGSIHGLTEGLHGFHVHEFGDNTAGSTSAGPRFVNQHLCGSHLVEALYLVCGERGFFYTPKTRRGIVEQCCTSICSLYQLENYCG

SEQ ID NO: 17 - protein, 117 aa, Artificial sequence
  Protein translated from synthetic DNA
MATKAVSVLKGDGPVQGIINFEQHESNGPVKVWGSIHGLTEGLHGFHVHEFGDNTAGSTSAGPRFVNQHLCGSHLVEALYLVCGERGFFYTPKTRRGIVEQCCTSICSLYQLENYCG

SEQ ID NO: 18 - protein, 120 aa, Artificial sequence
  Protein translated from synthetic DNA
MATHAVSVLKGDGPVQGIINFEQHESNGPVKVWGSIHGLTEGLHGFHVHEFGDNTAGSTSAGPRFVNQHLCGSHLVEALYLVCGERGFFYTPKTRREARGIVEQCCTSICSLYQLENYCG

SEQ ID NO: 19 - DNA, 354 bp, Artificial sequence
  Synthetic DNA
atggcgacgaaagccgtgagcgtgctgaagggcgacggcccagtgcagggcatcatcaatttcgagcagaaagaaagtaatggaccagtgaaggtgtggggaagcattcatggactgactgaaggcctgcatggattccatgttcatgagtttggagataatacagctggctctaccagtgcaggtccgaaatttgtgaaccagcatctgtgcggcagccatctggtggaagcgctgtatctggtgtgcggcgaacgcggcttcttttataccccgaaaacccgccgcggcattgtggaacagtgctgcaccagcatttgcagcctgtatcagctggaaaattattgcggctaa

SEQ ID NO: 20 - DNA, 354 bp, Artificial sequence
  Synthetic DNA
atggcgacgaaagccgtgagcgtgctgaagggcgacggcccagtgcagggcatcatcaatttcgagcagcatgaaagtaatggaccagtgaaggtgtggggaagcattcatggactgactgaaggcctgcatggattccatgttcatgagtttggagataatacagctggctctaccagtgcaggtccgaaatttgtgaaccagcatctgtgcggcagccatctggtggaagcgctgtatctggtgtgcggcgaacgcggcttcttttataccccgaaaacccgccgcggcattgtggaacagtgctgcaccagcatttgcagcctgtatcagctggaaaattattgcggctaa

SEQ ID NO: 21 - DNA, 363 bp, Artificial sequence
  Synthetic DNA
atggcgacgcatgccgtgagcgtgctgaagggcgacggcccagtgcagggcatcatcaatttcgagcagcatgaaagtaatggaccagtgaaggtgtggggaagcattcatggactgactgaaggcctgcatggattccatgttcatgagtttggagataatacagctggctctaccagtgcaggtccgcggtttgtgaaccagcatctgtgcggcagccatctggtggaagcgctgtatctggtgtgcggcgaacgcggcttcttttataccccgaaaacccgccgcgaagcccgcggcattgtggaacagtgctgcaccagcatttgcagcctgtatcagctggaaaactattgcggctaa

SEQ ID NO: 22 - DNA, 354 bp, Artificial sequence
  Synthetic DNA
atggcgacgaaagccgtgagcgtgctgaagggcgacggcccagtgcagggcatcatcaatttcgagcagaaagaaagtaatggaccagtgaaggtgtggggaagcattaaaggactgactgaaggcctgcatggattccatgttcatgagtttggagataatacagctggctctaccagtgcaggtccgaaatttgtgaaccagcatctgtgcggcagccatctggtggaagcgctgtatctggtgtgcggcgaacgcggcttcttttataccccgaaaacccgccgcggcattgtggaacagtgctgcaccagcatttgcagcctgtatcagctggaaaattattgcggctaa